European Patent Specification EP 3 539 372 B1, published December 6, 2023. Title: Wheat with increased resistant starch levels. Applicant: Arcadia Biosciences, Inc. Application US 13/894127. The sequence listing filed with the application follows.

SEQUENCE LISTING (58 sequences)

SEQ ID NO: 1 - DNA, 6114 bp, Triticum aestivum
caattaatatcgtccatcactcgggttccgcgctgcatttcggccggcgggttgagtgagatctgggccactgaccgactcactcgctcgctgcgcggggatggcgacgtttgcggtgtccggcgcgaccctcggtgtggcgcggcccgccggcgccggcggcggactgctgccgcgatccggctcggagcggaggggcggggtggacctgccgtcgctgctcctcaggaagaaggactcctctcgtacgcctcgctcgctcgctccaatctcccgtccatttttgccccccttctctctccctatctgcgcgcgcatggcctgttcgatgctgttccccagttgatctccatcaacgagagagatagctggattaggcgatcgcctgcgtcagtgtcacccaggccctggtgttatcacggctttgatcatctcctcccattctgatattttctcactctttcttctgttcttgctgtaactgcaagttgtagcattgtctcactattgtagtcatccttgcattgcaggcgccgtcctgagccgcgcggcctctccagggaaggtcctggtgcctgacggtgagagcgacgacttggcaagtccggcgcaacctgaagaattacaggtacacaccatcgtgccgggaaatcttcatacaatcgttattcacttaccaaatgccggatgaaaccaagccgcggaggcgtcaggttttgagcttcttctatcagcattgtgcagtactgcactgccttgtgcattttgttagccgtggccccgtgctggctcttgggccactgaaaactcagatggatgtgcattctagcaagaacttcacgaaataatgcactgtttgtggtttcgttagtctgctctacaattgctattttcgtgctgtagatacctgaagacatcgaggagcaaacggctgaagtaaacatgacaggggggactgcagaaaaacttgaatcttcagaaccgactcaaggcattgtggaaacaatcactgatggtgtaaccaaaggagttaaggaactagtcgtgggggagaaaccgcgagttgtcccaaaaccaggagatgggcagaaaatatacgagattgacccaacgctgaaagattttcggagccatcttgactaccggtaatgcctacccgctactttcgctcattttgaattaaggtcctttcgtcatgcaaatttggggaacatcaaagagacaaagactagggaccactatttcttacagttcccctcatggtctgagaatatgctgggacgtagatgtataattgatggctacaatttgctcataattacgatacaaataactgtctctgatcattgcaattacagagtggcaaactgattaaaatgtgatagatgggttatagattttactttgctaattcctctaccaaattcctggggaaaaaaatctaccagttgggcaacttagtttcttatctttgttgcctctttgttttggggaaaacacactgctaaatttgaatgattttgggtatgcctccgtggattcaacagatacagcgaatacaggagaattcgtgctgctattgaccaacatgaaggtggattggaagcattttctcgtggttatgaaaagcttggatttacccgcaggtaaatttaaagcttcagtattatgaagcgcctccactagtctacttgcatatcttacaagaaaatttataattcctgttttcgcctctcttttttccagtgctgaaggtattgtctagttgcatatcttataagaaaatttatgttcctgttttcccctattttccagtgctgaaggtatcacttaccgagaatgggctcctggagcgcatgtacgtcttttaagtcttaacagacaccttccaattcattgttaatggtcacactattcaccaactagcttactggacttacaacttagcttactgaatactgaccagttgctctaaatttatgatctggcttttgcatcctattacagtctgcagcattagtaggtgacttcaacaattggaatccgaatgcagatactatgaccagagtatgtctacagcttggcaatcttccacctttgcttcataactactgatacatctatttgtatttattttgctgtttgcacattccttaaagttgagcctcaactatatcatatcaaaatggtataatttgtcagtgtcttaagcttcagcctaaagattctactcaaattggtccatctttttgagattgaaaatgagtatattaaggatggatgaataggtgcaacactcccattctttggtagaaccttctgcattatgtgtgttttttcatctacaatgagcatatttccatgctatcagtgaaggtttgctcctattgatgccgatatttgatatgatcttttcaggatgattatggtgtttgggagattttcctccctaacaatgctgatggatccccagctattcctcatggctcacgtgtaaaggtaagctggccaattatttagttgaggatgtagcattttcgaactctgcccactaagggtccctttgcctttctgttttctagatacggatggatactccatctggtgtgaaggattcaatttctgcttggatcaagttctctgtgcaggctccaggtgaaataccattcaatggcatatattatgatccacctgaagaggtaagtatcgatctccattacattattaaatgaaatttccagtgttacggttttttaatacccatttcgtgtctcactgacatgtgagtcaagacaatactttagaatttggaagtgacatatgcattaattcaccttctaagggctaaggggcaagcaaccatggtgatgtttgtatgcttgtgtgtgacttaagatcttatagctcttttatgtgttctctgttggttaggatattccattttgaccttttgtgaccatttactaaggatatttacatgcaaatgcaggagaagtatgtcttccaacatcctcaacctaaacgaccagagtcactgaggatttatgaatcacacattggaatgagcagcccagtatgtcaataagttatttcacctgtttctggtctgatggtctattctatggattttttagttctgttatgtattgttaacatataacatggtgcattcacgtgacaacctcgattttattttctaatgttattgcaatagctcggtataatgtaaccatgttactagcttaagatggttagggtttcccacttaggatgcatgaaatatcgcattggagcatctccagcaagccatttttttgacggttaacagcaggagctctgcttttcattataggagagggaaatgctgtacagactgaagtcagtcagagcaaagtaacttagaatcatttatgggccaccctgcacagggcagaaggcaggcaggaacgatcctctacagccgtcggattgcctccatcagaggaatcctggccgttaatcatgctctggcccagtggtcagaatgcatcaaccagactgaggtgcttgcctccttattggtaaaggatgcagcggtacgagcctattgaacagatcctgttcaagtaaggccgttctccagcaagccatttcctagcttattaatgagagagagagagagaggggggggggtctgtattctgcgagcaattcaaaaacttccattgttctgaggtgtacgcattgtagggatctcccattatgaagaggatatagttaattctttgtaacctacttggaaacttgagtcttgcggcatcgctaatatattctatcatcacaatacttagaggatgcatctgaatattttagtgggatcttgcacaggaaccgaagataaattcatatgctaattttagggatgaggtgctgccaagaattaaaaggcttggatacaatgcagtgcagataatggcaatccaggagcattcatactatgcgagctttgggtattcacacaatccatttttttctgttcttttttctgtatgcgcctcttcacccatttggagctattacatcctaatgcttcgtgcacatagaatatttggatataattctttagtagacatatagtacaacaacagttggtatttctgacttgtatgaccattttattgttgttggcttgttccaggtaccatgttactaatttttttgcaccaagtagccgttttggaactccagaggacttaaaatccctgatcgatagagcacatgagcttggtttgcttgttcttatggatattgttcataggtaagtagtccaattaattttagctgctttactgtttatctggtattctaaatggcagggccgtatcgacgagtatttttccattctatataattgtgctacatgacttcttttttctcagatgtattaaaccagttggacatcaaatgtatttggtacatctagtaaactgacagtttcaaagaacatcgttttgtaatggcaacatgatttgatgccatagatgtggactgagaagttcagatgctatcaagaaaattaatcaactggccatgtactcgtggcactacatagagtttgcaagttggaaaactgacagcaatacctcactgataagtagctaggccccacttgccagcttcatattagatgttacttccctgttgaactcatttgaacatattacttaaagttcttcatttgtcctaagtcaaacttctttaagtttgaccaagtctactgaaaaatatatcaacatctacaacaccaaattggcttcattagattcacaatttttattttgtaatattagcacacctttgatgttgtagatatcagcacatttttctacagacttggtcaaatatagagaagtttgacttaggacaaatctagaacttcaatcaatttggatcagaggggatagtccatactggttgattatatccggtaacatcaaataatatagatagatgtcaacactttaacaaaaaaatcagaccttgtcaccaaatatgtatcagaccatctgtttgctttagccacttgttttcatatttatgtgtttgtacctaatctatttttacttctacttggtttggttgattttttttcagttgcattgcttcatcaatgattttgtgtaccctgcagtcattcatcaaataatacccttgacggcttgaatggtttcgatggcactgatacacattacttccacggtggtccacgtggccatcattggatgtgggattctcgtctattcaactatgggagttgggaagtatgtagctctgacttctgtcaccatatttggctaactgttcctgttaaatctgttcttacacatgtcgatattctattcttatgtaggtattgagattcttactgtcaaacgcgagatggtggcttgaagaatataagtttgatggatttcgatttgatggggtgacctccatgatgtatactcaccatggattacaagtaagtcatcaagtggtttcagtaacttttttagggcactgaaataattgctatgcatcataacatgtatcatgatcaggacttgtgctacggagtcttagatagttccctagtacgcttgtacaattttacctgatgagatcatggacgattcgaagtgattattatttatttttcttctaagtttgcttcttgttctagatgacatttactgggaactatggcgagtattttggatttgctactgatgttgacgcggtagtttacttgatgctggtcaacgatctaattcatggacttcatcctgatgctgtatccattggtgaagatgtaagtgcttacagtatttatgatttttaaccagttaagtagttttattttgggatcaggctgttactctttttgttaggggtaagatctctcttttcataacaatgctaatttataccttgtatgataatgcatcacttaggtaatttgaaaagtgcaaggccattcaagcttacgagcatattttttgatggctgtaatttatttgatagtatgcttgtttgggtttttcagtaaatgggagtgtgtgactaatgttgcattagaaatgggcaaccttgtca

SEQ ID NO: 2 - protein, 527 aa, Triticum aestivum
MATFAVSGATLGVARPAGAGGGLLPRSGSERRGGVDLPSLLLRKKDSSRAVLSRAASPGKVLVPDGESDDLASPAQPEELQIPEDIEEQTAEVNMTGGTAEKLESSEPTQGIVETITDGVTKGVKELVVGEKPRVVPKPGDGQKIYEIDPTLKDFRSHLDYRYSEYRRIRAAIDQHEGGLEAFSRGYEKLGFTRSAEGITYREWAPGAHSAALVGDFNNWNPNADTMTRDDYGVWEIFLPNNADGSPAIPHGSRVKIRMDTPSGVKDSISAWIKFSVQAPGEIPFNGIYYDPPEEEKYVFQHPQPKRPESLRIYESHIGMSSPEPKINSYANFRDEVLPRIKRLGYNAVQIMAIQEHSYYASFGYHVTNFFAPSSRFGTPEDLKSLIDRAHELGLLVLMDIVHSHSSNNTLDGLNGFDGTDTHYFHGGPRGHHWMWDSRLFNYGSWEVLRFLLSNARWWLEEYKFDGFRFDGVTSMMYTHHGLQMTFTGNYGEYFGFATDVDAVVYLMLVNDLIHGLHPDAVSIGED

SEQ ID NO: 3 - DNA, 10219 bp, Triticum aestivum
tgagatctgggccactgaccgactcactcgctgcgcggggatggcgacgttcgcggtgtccggcgcgaccctcggtgtggcgcggcccgccagcgccggcggcggactgctgcgatccggctcggagcggaggggcggggtggacttgccgtcgctgctcctcaggaagaaggactcctctcgtacgcctcgctccctccaatctccccgtctgtttttgggcccccttctctctccctcgcctctctgcgcgcgcatggcctgttcgatgctgttccccagttgatctccatgaacgagagagatagctggattaggcgatcgcctcaggccctggtgttaccacggctttgatcatctcctcctttcatgctgatattttctcactctttcttctgttcttgctgtaactgcaagttgtagcatttttttggcgaataagttgtagcattgtctcactattgtactcatccttgcatttgcaggcgccgtcctgagccgcgcggcctctccagggaaggtcctggtgcctgacggtgagagcgacgacttggcggccactccagcgcaacccgaagaattacaggtacacaccgtcgtgccggaaaatcttcatgcacccgttattcacttaccaaatatcggatgaaccaagccgcggaggcatcaggtttcaagcttcttctatcagcattgtgcactacttcactgccttgtgcagtttgttagctgtggccccgcgctggctcttgggccactgaaaactcagatggatgtgcattctagcaagaacttcacaaaataatgcactgtttgtggtttcgttagtctgctctacaattgctatttttcgtgtgctgtagatacctgaagatatcgaggagcaaacggctgaagtgaacatgacaggggggactgcagagaaacttcaatattcagaaccgactcagggcattgtggaaacaatcactgatggtgtaaccaaaggagttaaggaactagtcgtgggggagaaaccgcgagttgtcccaaaaccaggagatgggcagaaaatatacgagattgacccaacgctgaaagattttcggagccatcttgactaccggtaatgcctacccgctaatttcgctcattttgaattaaggtcctttcatcatgcaaatttggggaacatcaaagaggcaaagactagggaccactgtttcatacagttcccctcatggtctgagaatatgctgggaagtatatgtataattgctggctacaattggctcataattgcaatacaaataactgtctccgatcattacaattacagagtggcaaactgatgaaaatgtggtggatgggttatggattttactttgctaattcctctaccaaattcctggggaaaaaatctaccagttgggcaacttagtttcttatctttgttgcctttttgttttggggaaaacacactgctaaatttgaatgattttgggtatgccttggtggattcaacagatacagcgaatacaagagaattcgtgctgctattgaccaacatgaaggtggattggaagcattttctcgtggttatgaaaagcttggatttacccgcaggtaaatttaaagctttactatgaaacgcctccactagtctaattgcatatcttgtaagaaaatttataattcctgttttcccctctcttttttccagtgctgaaggtatcatctaattgcttatcttataagaaaatttataattcctgtttccccccctctttttccagtgctgaaggtatcacttaccgagaatgggctcctggagcgcatgtacgtcttaacagacaccttctaatctattgttaatggtcactattcaccaactagcttactgaacttacaaaatagcttactgaatactgaccagttactctaaatttatgatctggcttttgcatcctgttacagtctgcagcattagtaggtgacttcaacaattggaatccaaatgcagatactatgaccagagtatgtctacagcttggcaatcttccacctttgcttcgtaactactgatacatctatttgtatttatttaactgtttgcacgttcgttaaagttgagcctcaactatatcataccaaaatggtataatttgtcagtgtcttaagcttcagcctaaagatcctactgaatttagtccatccttttgagattgaaaatgagtatattaagggtgattgaatacttgcaacactcccattttttggtagaaccttttgcattatgtgtgcttttccatccacaatgagcatatttccatgttatcagtgaaggtttgctcctattgatgccgatatttgatatgatctttcgatcttttcaggatgattatggtgtttgggagatcttcctccctaacaatgctgatggatccccagctattcctcatggctcacgtgtaaaggtaatctggccaattatttagtcgaggatgtaacattttcgaactctgcctactaagggtcccttttcctctctattttctagatacggatggatactccatctggtgtgaaggattcgatttctgcttggatcaagttctctgtgcaggctccaggtgaaataccattcaatggcatatattatgatccacctgaagaggtaagtatcaatctatgttacattattaaatggaatttccagtgttacagttttttgatacccacttcatgtctcactgacatgtgagtcaagacaatactttcgaatttggaagtgacatatgcattaattcaccttctaagggctaaggggcaaccaaccatggtgatgtgtgtatgcttgtgtgacttaagatcttatagctcttttatatgttctctgttggttaggacattccattttgaccttttgtgaccatttactaaggatattttacatgcaaatgcaggagaagtatgtcttccaacatcctcaacctaaacgaccagagtcactaaggatttatgaatcacacattggaatgagcagcccggtatgtcaataagttatttcacctgtttccggtctgatggtttattctatggattttctagttctgttatgtactgttaacataccacacggtgcattcacgtgacaacctcgattttattttctaatgtcttcatattggaaaatgcacaactttgcttcctctttgtctgatcgtttttttgtctctaagatttccattgcatttcgaggtagcgggcatgtgaaagtcgaatctgaatattttttgtcagagcacagttatattaaatgccattgttgttgcaatagcttggtataatgtagccatgttactagcttaagaaatatcgcattggagcatctccagcaagccatttcctaccttattactgagggggggggggggggggagcggggttctgtattctgcgagcgattcaaaacttccactgttctgaggtgtacgtactgtagggatctcccattatgaagaggacatagttaactttttgtaacctacttggaaacttgagtcttgatgcatcgctactatatactatcatcacaatacttagaggatgcatctgaatattttagcgtgatcttgcacaggaaccgaagataaattcatatgctaattttagggatggggtgctgccaagaattaaaaggcttggatacaatgcagtgcagataatggcaatccaggagcattcatactatgcaagctttgggtattcatacagtccatctttttctgttttttttttctgtatgtgcctcttcacccatttcgagccattacatcctaatgcttcgtgcacataaaatacttggatataattctttattagacatatagtacaacaccacttagtatttctgacttgtatgatcattttattgttgttggcttgttacaggtaccatgttactaatttttttgcaccaagtagccgttttggaactccagaggacttaaaatccttgatcgatagagcacatgagcttggtttgcttgttcttatggatattgttcataggtaatcagtccaatttaattttagttgctttactgtttatctggtattgtaaatggcagggccctatcgtcgaatatttttccaatctatataattgtgctacatgacttattttttctcagatgtattaaaccagttggatattaaatgtatttggtacatctagtaaactgacagtttcatagaattgtgttgtaatggcaacacaatttgatggcatagatgtggactgagaagttcagatgctatcagtaattaattaactggccatgtactcgtggaactacatagagtttgcaagttggaaaactgacagcaatacctcactgataagtgtccaggccacacttgccagcttcatattagatgttacttccctgttgaactcctttgaacatatcacttaaagttcttcaattgtcctaagtcaaacttctttgactttggccaagtctattgaaaaatatgtcaacatctacagcaccaaattagtttcataatttttattttgttatattagcacgttttttatgctgtagatatcagcacatttttctatagacttggtcaaatatagagaagtttgacttaggacaaatcagaacttcaagcaatttggatcagagggaatagtccatactgcttgattatattttcccaaaggagggagtgaggagcttgacttcggtatcatcaaatgatattgatagatgtcaacattttaacaaaaaatcagaccttgtcaccaaatatgcatcagaccatctgtttgcttaggcacttgctttcatatttatgtgtttgtaactaatctacttttccttctacttggtttgattgattctatttcagttgcattgcttcatcaatgattttgtgtaccctgcagtcattcgtcaaataatacccttgacggtttgaatggtttcgatggcactgatacacattacttccacggtggtccacgtggccatcattggatgtgggattctcgtctgttcaactatgggagttgggaagtatgtagctgcgacttctgtcaccatgtttggctaactgttcctgccaatctgttcttacacgtgtcaatattctattcttatacaggtattaagattcttactgtcaaacgcgagatggtggcttgaagaatataagtttgatggatttcgatttgatggggtgacctccatgatgtatactcaccatggattacaagtaagtcatcaagtggtttcagtaacttcttcagggcactgaaacaattgctatgcatcataacatgtatcatgatcagtacttatgctacggagtcttagatagttccctagtatgcttgtacaattttacctgatgagatcatggaagattggaagtgattgttattatttttccttctaagtttgcttcttgttctagatgacatttactgggaactatggcgagtattttggatttgccactgatgttgatgcggtggtatacttaatgctggtcaacgatctaattcatggactttatcctgatgctgtatccattggtgaagatgtaagtgcttacagtatttatgttttttagtattttattttggggatcaagctgttactactctttttgttagggtaaaatctgtcttttcataagaatgctaatttatactccctccgtctggaaatacttgtcggaggaatgaatgtatctagacgtattttagttctagatacatccatttttatgcatttctccgtcaagtatttccggacggagggagtaccttgtatggtaatgcatcacataggtaatttgagaagtgcaagggcattcaagctgacaagcatatttgttgatggctgtaatttatttgatagtatgcttgtttggatttttcagtaagtgtgagtgtgtgagtaatgttatattatttatttacttgcggaagaaatgggcaaccttgtcaattgcttcagaagactaacttagattccataaatgctgtggaaatgagaggctattcccaaggacacgaaattatacgtcagtgtgttacgcacatgtatttgtaagagcaagagcaacatggtttaacttaaattcctgcactgctatggaatctcactgtatgttgttagtgtacgcatccacaaacaagtaatcctgagctttcaactcacgagaaaataggaggctccacttctgccagcattagctgttcacagttctaatttgtgtaactctgaaattgttcaggtcagtggaatgcctacattttgcatccctgttccagatggtggtgttggttttgactatcgcctgcatatggctgtagcagataaatggatcgaactcctcaagtaagtgcaggaatattggtgattacatgcgcacaatgatctactccctctgtcccataatgtaagatgttttttgacactagtgtagtgtcaaaaaacgtcctatattatgggaaggagggagtagttcacaatttctaaattgtaaaaagaaaaatatgtatgtgaatagctagacatttccctggtatcagcttcaacacaagaagatttatcaaatacatgatttaaatagcaaatttcggaaatgtaatggctagtgtctttatgctggatattgtacatggcgctgtagcaggtgagtcaataaagctagcgatattttcagaaacaaaataatcatttatatctgtatatggggaaagtgggggtatagatggtggtcattaatcgtgttcactttttgtcctgtataagcacaggcagtaggtaataaatttagccagataaaataaatcgttattaggtttacaaaaggaatacagagggtcatgtagcatatctagttgtagttattgtaaaggctgacaagaggttcagtaaaaaaaactttatgttgatcccgggtatgcaagaacgcgagtaaagctcaaacatttatagtggttgctgttgcttgctgtatacttgtatctgcgcatatatgaaattactactacacagctgccaatctgccatgatctgtgttttgctttgtgctatttaaattttaaatgctaactcaataaatggcaataataaactaactattcaaccaatttgatggatatcagagatttcttccctcctttagtaacattgtgctcctgctgctgttctctaccgttacaaaagctgtttttccatttttcgcatcattatttttgtgtgtgagtaatttaagcatgtcctttgaagctgtgagctgttggtacttagtacattcttggtagtgtccaaatatgctgcagtctaatttagcatttctataacacaggcaaagtgacgaatcttggaaaatgggtgatattgtgcacaccctaacaaatagaaggtggcttgagaagtgcgtcacttatgcagaaagtcatgatcaagcactagttggtgacaagactattgcattctggttgatggataaggtactagctgttacttttggatcaaaagaatcacataagatttgtctcatcagattgctcatgttttcttgtgataaagatttggccccctcacccatcaccagctatttcccaactgtcacttgagcaaaacgtgccatgtggcactgtggtggcttgtgaactttgacagttaatgttgcaaatttctgttcttatttatttgattcttatgttatcgttcatttattcctcaaaaaatgttatcgttcatttgctcattcctttccgagaccagccgaagtcacgtgtagccatgtgatctgccatctgaatcttgagcaaattttatgaagaggctaaagtcgaacggattatttgcttgaatttataaatatacagacgtataatcacctggtgctttctgaaatgattaccatagtgcctgaaggctgaaatagttttggcgtttcctggacgacgcccaaaggagtgaattttattgggtagatttctggctgagccctggttacaacatacattttggagatatgcttaataacaaatctgggtgtttggtcacgagtctgcatctacatgctccttgggttttattatggcgtcatctttgtaactagtggcacccctaaggaaacattcaaaaggaaactgttacatcattctagtcaggaccaccgtactaagagcaaaattctgttccaattttatgagtttttgagactccaaaatgaacataagtgtctcatattttgctaattaactacagatgtttttatatcactttagtttttatttcaggacagttgatacttggtactgtgctgtaagcattgatccgacacagaacagcatgaacatttcgagctctctttgtgcaggatatgtatgatttcatggctctggatagaccttcaactcctcgcattgatcgtggcatagcattacataaaatgatcaggcttgtcaccatgggtttaggtggcgaaggctatcttaacttcatgggaaatgagtttgggcatcctggtcagtctttacaacattattgcattctgcatggttgtgatttactgtaatttgaaccatgctttgttttcacattgtatgtattatgtaatctgttgcttccaaggaggaagttaacttctatttacttggcagaatggatagattttccaagaggtccgcaaactcttccaaccggcaaagttctccctggaaataacaatagttatgataaatgccgccgtagatttgatcttgtaagttttagctgtgctcttacgttccctcactagatctttattggctatttatttcttgatgaaatcataatgtttgttgatcaacattgcttttgtagttttgtagacgttaacataaatatgtgttaagagttattgatcattaagaatatcatgattttttttgtagggagatgcagattttcttagatatcgtggtatgcaagagttcgaccaggcaatgcagcatcttgaggaaaaatatggggtatgtcagtatgtcactggtttgtctttgttgcatagcaagtcacagtttaacgccagtctcttcaaatggtcaaaaagtgtagaattaattcctgtaatgagatgaaaactgcgcaaaggcgggagctggaattgcttttcaccaattaaaactattttcttaagcgattgtgtattgatacctataccaacactgacaatgtaactgcagtttatgacatctgagcaccagtatgtttcacggaaacatgaggaagataaggtgatcatcttcgaaagaggagatttggtatttgttttcaacttccactggagcaatagcttttttgactaccgtgttgggtgttccaagcctgggaagtacaaggtatgcttgccttttcattgcccacccttcaccagtagggttagtgggggcttctacaacttttaattccacatgtagagtttgttgttcgtgcagctatcaatataaagaataggataatttgtaaagaaaagaatttgttgctcgagatgttgtagtcatataacatccccgaagcacatctactattcattcatattatctacttaagggtttgttacaatctttgtactcagttggactcactctaatactggaactatttaccgaatctaccctaatcatcctagcagttttagagcagccccatttggacagtccactgggtttagttggtttgtgacagtttctgctatttcttaatcaggtggccttagactccgacgatgcactctttggtggattcagcaggcttgatcatgatgtcgactacttcacaaccgtaagtctgggctcaagcgtcacttgactcgtctagactcaactgcttacaaatctgaatcaacctcccatttgctgatgcccttgcaggaacatccgcatgacaataggccgcgctctttcttggtgtacactcctagcagaactgcggtcgtgtatgcccttacagagtaagaaccagcagcggcttgttacaaggcaaagagagaactccagggagctcgtggattgtgagcgaagcgacgggcaactgcgtgaggctgctctaagcgccatgactgggaggggatcgtgcctcttcccctgatgccaggaggatcagatggataggtagcttgttgggaaaaatatggggtatgtcagtatgtcact

SEQ ID NO: 4 - protein, 823 aa, Triticum aestivum
MATFAVSGATLGVARPASAGGGLLRSGSERRGGVDLPSLLLRKKDSSRAVLSRAASPGKVLVPDGESDDLAATPAQPEELQIPEDIEEQTAEVNMTGGTAEKLQYSEPTQGIVETITDGVTKGVKELVVGEKPRVVPKPGDGQKIYEIDPTLKDFRSHLDYRYSEYKRIRAAIDQHEGGLEAFSRGYEKLGFTRSAEGITYREWAPGAHSAALVGDFNNWNPNADTMTRDDYGVWEIFLPNNADGSPAIPHGSRVKIRMDTPSGVKDSISAWIKFSVQAPGEIPFNGIYYDPPEEEKYVFQHPQPKRPESLRIYESHIGMSSPEPKINSYANFRDGVLPRIKRLGYNAVQIMAIQEHSYYASFGYHVTNFFAPSSRFGTPEDLKSLIDRAHELGLLVLMDIVHSHSSNNTLDGLNGFDGTDTHYFHGGPRGHHWMWDSRLFNYGSWEVLRFLLSNARWWLEEYKFDGFRFDGVTSMMYTHHGLQMTFTGNYGEYFGFATDVDAVVYLMLVNDLIHGLYPDAVSIGEDVSGMPTFCIPVPDGGVGFDYRLHMAVADKWIELLKQSDESWKMGDIVHTLTNRRWLEKCVTYAESHDQALVGDKTIAFWLMDKDMYDFMALDRPSTPRIDRGIALHKMIRLVTMGLGGEGYLNFMGNEFGHPEWIDFPRGPQTLPTGKVLPGNNNSYDKCRRRFDLGDADFLRYRGMQEFDQAMQHLEEKYGFMTSEHQYVSRKHEEDKVIIFERGDLVFVFNFHWSNSFFDYRVGCSKPGKYKVALDSDDALFGGFSRLDHDVDYFTTEHPHDNRPRSFLVYTPSRTAVVYALTE

SEQ ID NO: 5 - DNA, 11475 bp, Aegilops tauschii
  misc_feature (4795)..(4795): n is a, c, g, or t
  misc_feature (4973)..(4973): n is a, c, g, or t
  misc_feature (5078)..(5079): n is a, c, g, or t
  misc_feature (5082)..(5082): n is a, c, g, or t
  misc_feature (7010)..(7010): n is a, c, g, or t
  misc_feature (7327)..(7327): n is a, c, g, or t
  misc_feature (7381)..(7381): n is a, c, g, or t
  misc_feature (7384)..(7384): n is a, c, g, or t
  misc_feature (7819)..(7819): n is a, c, g, or t
  misc_feature (8189)..(8189): n is a, c, g, or t
agaaacacctccattttagattttttttttgttcttttcggacggtgggtcgtggagagattagcgtctagttttcttaaaagaacaggccatttaggccctgctttacaaaaggctcaaccagtccaaaacgtctgctaggatcaccagctgcaaagttaagcgcgagaccaccaaaacaggcgcattcgaactggacagacgctcacgcaggagcccagcaccacaggcttgagcctgacagcggacgtgagtgcgtgacacatggggtcatctatgggcgtcggagcaaggaagagagacgcacatgaacaccatgatgatgctatcaggcctgatggagggagcaaccatgcaccttttcccctctggaaattcatagctcacacttttttttaatggaagcaagagttggcaaacacatgcattttcaaacaaggaaaattaattctcaaaccaccatgacatgcaattctcaaaccatgcaccgacgagtccatgcgaggtggaaacgaagaactgaaaatcaacatcccagttgtcgagtcgagaagaggatgacactgaaagtatgcgtattacgatttcatttacatacatgtacaaatacataatgtaccctacaatttgttttttggagcagagtggtgtggtcttttttttttacacgaaaatgccatagctggcccgcatgcgtgcagatcggatgatcggtcggagacgacggacaatcagacactcaccaactgcttttgtctgggacacaataaatgtttttgtaaacaaaataaatacttataaacgagggtactagaggccgctaacggcatggccaggtaaacgcgctcccagccgttggtttgcgatctcgtcctcccgcacgcagcgtcgcctccaccgtccgtccgtcgctgccacctctgctgtgcgcgcgcacgaagggaggaagaacgaacgccgcacacacactcacacacggcacactccccgtgggtcccctttccggcttggcgtctatctcctctcccccgcccatccccatgcactgcaccgtacccgccagcttccacccccgccgcacacgttgctcccccttctcatcgcttctcaattaatatctccatcactcgggttccgcgctgcatttcggccggcgggttgagtgagatctgggcgactggctgactcaatcactacgcggggatggcgacgttcgcggtgtccggcgcgactctcggtgtggcgcgggccggcgtcggagtggcgcgggccggctcggagcggaggggcggggcggacttgccgtcgctgctcctcaggaagaaggactcctctcgtacgcctcgctctctcgaatctcccccgtctggctttggctccccttctctctcctctgcgcgcgcatggcctgttcgatgctgttccccaattgatctccatgagtgagagagatagctggattaggcgatcgcgcttcctgaacctgtattttttcccccgcggggaaatgcgttagtgtcacccaggccctggtgttaccacggctttgatcattcctcgtttcattctgatatatattttctcattctttttcttcctgttcttgctgtaactgcaagttgtggcgttttttcactattgtagtcatccttgcattttgcaggcgccgtcctgagccgcgcggcctctccagggaaggtcctggtgcctgacggcgagagcgacgacttggcaagtccggcgcaacctgaagaattacaggtacacacactcgtgccggtaaatcttcatacaatcgttattcacttaccaaatgccggatgaaaccaaccacggatgcgtcaggtttcgagcttcttctatcagcattgtgcagtactgcactgccttgttcattttgttagccttggccccgtgctggctcttgggccactgaaaaaatcagatggatgtgcattctagcaagaacttcacaacataatgcaccgtttggggtttcgtcagtctgctctacaattgctatttttcgtgctgtagatacctgaagatatcgaggagcaaacggcggaagtgaacatgacaggggggactgcagagaaacttcaatcttcagaaccgactcagggcattgtggaaacaatcactgatggtgtaaccaaaggagttaaggaactagtcgtgggggagaaaccgcgagttgtcccaaaaccaggagatgggcagaaaatatacgagattgacccaacactgaaagattttcggagccatcttgactaccggtaatgcctacccgctgctttcgctcattttgaattaaggtcctttcatcatgcaaatttggggaacatcaaagagacaaagactagggaccaccatttcatacagatcccttcgtggtctgagaatatgctgggaagtaaatgtataattgatggctacaatttgctcaaaattgcaatacgaataactgtctccgatcattacaattaaagagtggcaaactgatgaaaatgtggtggatgggttatagattttactttgctaattcctctaccaaattcctaggggggaaatctaccagttgggaaacttagtttcttatctttgtggcctttttgttttggggaaaacacattgctaaattcgaatgattttgggtatacctcggtggattcaacagatacagcgaatacaagagaattcgtgctgctattgaccaacatgaaggtggattggaagcattttctcgtggttatgaaaagcttggatttacccgcaggtaaatttaaagctttattattatgaaacgcctccactagtctaattgcatatcttataagaaaatttataattcctgttttcccctctcttttttccagtgctgaaggtatcgtctaattgcatatcttataagaaaatttatattcctgttttcccctattttccagtgctgaaggtatcacttaccgagaatgggctcctggagcgcatgttatgttcttttaagttccttaacgagacaccttccaatttattgttaatggtcactattcaccaactagcttactggacttacaaattagcttactgaatactgaccagttactataaatttatgatctggcttttgcaccctgttacagtctgcagcattagtaggtgacttcaacaattggaatccaaatgcagatactatgaccagagtatgtctacagcttggcaattttccacctttgcttcataactactgatacatctatttgtatttatttagctgtttgcacattccttaaagttgagcctcaactacatcatatcaaaatggtataatttgtcagtgtcttaagcttcagcccaaagattctactgaatttagtccatctttttgagattgaaaatgagtatattaaggatgaatgaatacgtgcaacactcccatctgcattatgtgtgcttttccatctacaatgagcatatttccatgctatcagtgaaggtttgctcctattgatgcagatatttgatatggtcttttcaggatgattatggtgtttgggagattttcctccctaacaacgctgatggatcctcagctattcctcatggctcacgtgtaaaggtaagctggccaattatttagtcgaggatgtagcattttcgaactctgcctactaagggtcccttttcctctctgttttttagatacggatggatactccatccggtgtgaaggattcaatttctgcttggatcaagttctctgtgcaggctccaggtgaaatacctttcaatggcatatattatgatccacctgaagaggtaagtatcgatctacattacattattaaatgaaatttccagtgttacagttttttaatacccacttcttactgacatgtgagtcaagacaatacttttgaatttggaagtgacatatgcattaattcaccttctaagggctaaggggcaaccaaccttggtgatgtgtgtatgcttgtgtgtgacataagatcttatagctcttttatgtgttctctgttggttaggatattccattttggccttttgtgaccatttactaaggatatttacatgcaaatgcaggagaagtatgtcttccaacatcctcaacgtaaacgaccagagtcactaaggatttatgaatcacacattggaatgagcagcccggtatgtcaataagttatttcacctgtttctggtctgatggtttattctatggattttctagttctgttatgtactgttaacatattacatggtgcattcacttgacaacctcgattttattttctaatgtcttcatattggcaagtgcaaaactttgcttcctctttgtctgcttgttcttttgtcttctgtaagatttccattgcatttggaggcagtgggcatgtgaaagtcatatctattttttttttgtcagagcatagttatatgaattccattgttgttgcaatagctcggtataatgtaaccatgttactagcttaagatttcccacttaggatgtaagaaatattgcattggagcgtctccagcaagccatttcctaccttattaatgagagagagacaaggggggggggggggggggggttcccttcattattctgcgagcgattcaaaaacttccattgttctgaggtgtacgtactgcagggatctcccattatgaagaggatatagttaattctttgtaacctacttggaaacttgagtcttgaggcatcgctaatatatactatcatcacaatacttagaggatgcatctgaanattttagtgtgatcttgcacaggaaccgaagataaattcatatgctaattttagggatgaggtgttgccaagaattaaaaggcttggatacaatgcagtgcagataatggcaatccaggagcattcatactatgcaagctttgggtattcacacaatccatttttttctgtatacacntcttcacccatttggagctattacatcctaatgcttcatgcacataaaatatttggatataatcctttattagatatatagtacaactacacttagtattctgannaanaagatcattttattgttgttggcttgttccaggtaccatgttactaatttttttgcaccaagtagccgttttggaactccagaggacttaaaatccttgatcgatagagcacatgagcttggtttgcttgttcttatggatattgttcataggtaattagtccaatttaattttagctgttttactgtttatctggtattctaaagggaaattcaggcaattatgatacattgtcaaaagctaagagtggcgaaagtgaaatgtcaaaatctagagtggcataaggaaaattggcaaaaactagagtggcaaaaataaaattttcccatcctaaatggcagggccctatcgccgaatatttttccattctatataattgtgctacgtgacttcttttttctcagatgtattaaaccagttggacatgaaatgtatttggtacatgtagtaaactgacagttccatagaatatcgttttgtaatggcaacacaatttgatgccatagatgtggattgagaagttcagatgctatcaatagaattaatcaactggccatgtactcgtggcactacatatagtttgcaagttggaaaactgacagcaatacctcactgataagtggccaggccccacttgccagcttcatactagatgttacttccctgttgaattcatttgaacatattacttaaagttcttcatttgtcctaagtcaaacttctttaagtttgaccaagtctattggaaaatatatcaacatctacaacaccaaattactttgatcagattaacaatttttattttattatattagcacatctttgatgttgtagatatcagcacatttttctatagacttggtcaaatatagagaagtttgacttaggacaaatctagaacttcaatcaatttggatcagagggaacatcaaataatatagatagatgtcaacacttcaacaaaaaaatcagaccttgtcaccatatatgcatcagaccatctgtttgctttagccacttgctttcatatttatgtgtttgtacctaatctacttttccttctacttggtttggttgattctatttcagttgcattgcttcatcaatgattttgtgtaccctgcagtcattcgtcaaataatacccttgacggtttgaatggtttcgatggcactgatacacattacttccacggtggtccacgcggccatcattggatgtgggattctcgtctattcaactatgggagttgggaagtatgtagctctgacttctgtcaccatatttggctaactgttcctgttaatctgttcttacacatgttgatattctattcttatgcaggtattgagattcttactgtcaaacgcgagatggtggcttgaagaatataagtttgatggatttcgatttgatggggtgacctccatgatgtatactcaccatggattacaagtaagtcatcaagtggtttcagtaacttttttagggcactgaaacaattgctatgcatcataacatgtatcatgatcaggacttgtgctacggagtcttagatagttccctagtatgcttgtacaattttacctgatgagatcatggaagattggaagtgattattatttattttctttctaagtttgtttcttgttctagatgacatttactgggaactatggcgaatattttggatttgctactgatgttgatgcggtagtttacttgatgctggtcaacgatctaattcatggactttatcctgatgctgtatccattggtgaagatgtaagtgcttacagtatttatgatttttaactagttaagtagttttattttggggatcagtctgttacactttttgttaggggtaaaatctctcttttcataacaatgctaatttataccttgtatgataatgcatcacttangtaatttgaaaagtgcaagggcattcaagcttacgagcatattttttgatggctgtaatttatttgatagtatgcttgtttgggtttttcaataagtgggagtgtgtgactaatgttgtattatttatttaattgcggaagaaatgggcaaccttgtcaattgcttcagaaggctaactttgattccataaacgctttggaaatgagaggctattcccaaggacatgaattatacttcagtgtgttctgtacatgtatttgtaatagtggtttaacttaaattcctgcactgctatggaatctcactgtatgttgtnagtgtacacatccacaaacaagtaatcctgagctttcaactcatgagaaaatangangtccgcttctgccagcattaactgttcacagttctaatttgtgtaactgtgaaattgttcaggtcagtggaatgcctacattttgcatccctgttccagatggtggtgttggttttgactaccgcctgcatatggctgtagcagataaatggattgaactcctcaagtaagtgcaggaatattggtgattacatgcgcacaatgatctagattacattttctaaatggtaaaaaggaaaatatgtatgtgaatatctagacatttgcctgttatcagcttgaatacgagaagtcaaatacatgatttaaatagcaaatctcggaaatgtaatggctagtgtctttatgctgggcagtgtacattgcgctgtagcaggccagtcaacacagttagcaatattttcagaaacaatattatttatatccgtatatgangaaagttagtatataaactgtggtcattaattgtgttcaccttttgtcctgtttaaggatgggcagtaggtaataaatttagccagataaaataaatcgttattaggtttacaaaaggaatatacagggtcatgtagcatatctagttgtaattaatgaaaaggctgacaaaaggctcggtaaaaaaaactttatgatgatccagatagatatgcaggaacgcgactaaagctcaaatacttattgctactacacagctgccaatctgtcatgatctgtgttctgctttgtgctatttagatttaaatactaactcgatacattggcaataataaacttaactattcaaccaatttggtggataccaganatttctgccctcttgttagtaatgatgtgctccctgctgctgttctctgccgttacaaaagctgttttcagttttttgcatcattatttttgtgtgtgagtagtttaagcatgttttttgaagctgtgagctgttggtacttaatacattcttggaagtgtccaaatatgctgcagtgtaatttagcatttctttaacacaggcaaagtgacgaatcttggaaaatgggcgatattgtgcacaccctaacaaatagaaggtggcttgagaagtgtgtaacttatgcagaaagtcatgatcaagcactagttggtgacaagactattgcattctggttgatggataaggtactagctgttacttttggacaaaagaattactccctccgttcctaaatataagtctttgtagagattccactatggaccacatagtatatagatgcattttagagtgtagattcactcattttgcttcgtatgtagtccatagtgaaatctctacagagacttatatttaggaacggagggagtacataattgatttgtctcatcagattgctagtgttttcttgtgataaagattggctgcctcacccatcaccagctatttcccaactgttacttgagcagaatttgctgaaaacgtaccatgtggtactgtggcggcttgtgaactttgacagttatgttgcaattttctgttcttatttatttgattgcttatgttaccgttcatttgctcattcctttccgagaccagccaaagtcacgtgttagctgtgtgatctgttatctgaatcttgagcaaattttattaataggctaaaatccaacgaattatttgcttgaatttaaatatacagacgtatagtcacctggctctttcttagatgattaccatagtgcctgaaggctgaaatagttttggtgtttcttggatgccgcctaaaggagtgatttttattggatagattcctggccgagtcttcgttacaacataacattttggagatatgcttagtaacagctctgggaagtttggtcacaagtctgcatctacacgctccttgaggttttattatggcgccatctttgtaactagtggcacctgtaaggaaacacattcaaaaggaaacggtcacatcattctaatcaggaccaccatactaagagcaagattctgttccaattttatgagtttttgggactccaaagggaacaaaagtgtctcatattgtgcttataactacagttgtttttataccagtgtagttttattccaggacagttgatacttggtactgtgctgtaaattatttatccgacatagaacagcatgaacatatcaagctctctttgtgcaggatatgtatgatttcatggctctggataggccttcaactcttcgcattgatcgtggcatagcattacataaaatgatcaggcttgtcaccatgggtttaggtggtgaaggctatcttaacttcatgggaaatgagtttgggcatcctggtcagtctttacaacattattgcattctgcatgattgtgatttactgtaatttgaaccatgcttttctttcacattgtatgtattatgtaatctgttgcttccaaggaggaagttaacttctatttacttggcagaatggatagattttccaagaggcccacaaactcttccaaccggcaaagttctccctggaaataacaatagttatgataaatgccgccgtagatttgatcttgtaagttttagctgtgctattacattccctcactagatctttattggccatttatttcttgatgaaatcataatgtttgttaggaaagatcaacattgcttttgtagttttgtagacgttaacataagtatgtgttgagagttgttgatcattaaaaatatcatgattttttgcagggagatgcagattttcttagatatcgtggtatgcaagagttcgatcaggcaatgcagcatcttgaggaaaaatatggggtatgtcactggtttgtctttgttgcataacaagtcacagtttaacgtcagtctcttcaagtggtaaaaaaagtgtagaattaattcctgtaatgagatgaaaactgtgcaaaggcggagctggaattgcttttcaccaaaactattttcttaagtgcttgtgtattgatacatataccagcactgacaatgtaactgcagtttatgacatctgagcaccagtatgtttcacggaaacatgaggaagataaggtgatcatcctcaaaagaggagatttggtatttgttttcaacttccactggagcaatagcttttttgactaccgtgttgggtgttccaagcctgggaagtacaaggtatgcttgccttttcattgtccacccttcaccagtagggttagtgggggcttctacaacttttaattccacatggatagagtttgttggtcgtgcagctatcaatataaagaatagggtaatttgtaaagaaaagaatttgctcgagctgttgtagccataggaaggttgttcttaacagccccgaagcacataccattcattcatattatctacttaagtgtttgtttcaatctttatgctcagttggactcggtctaatactagaactattttccgaatctaccctaaccatcctagcagttttagagcagccccatttggacaattggctgggtttttgttagttgtgacagtttctgctatttcttaatcaggtggccttggactctgacgatgcactctttggtggattcagcaggcttgatcatgatgtcgactacttcacaaccgtaagtctgggctcaagcgtcacttgactcgtcttgactcaactgcttacaaatctgaatcaacttcccaattgctgatgcccttgcaggaacatccgcatgacaacaggccgcgctctttctcggtgtacactccgagcagaactgcggtcgtgtatgcccttacagagtaagaaccagcagcggcttgttacaaggcaaagagagaactccagagagctcgtggatcgtgagcgaagcgacgggcaacggcgcgaggctgctccaagcgccatgactgggaggggatcgtgcctcttccccagatgccaggaggagcagatggataggtagcttgttggtgagcgctcgaaagaaaatggacgggcctgggtgtttgttgtgctgcactgaaccctcctcctatcttgcacattcccggttgtttttgtacatataactaataattgcccgtgcgctcaacgtgaaaatcc

SEQ ID NO: 6 - protein, 819 aa, Aegilops tauschii
MATFAVSGATLGVARAGVGVARAGSERRGGADLPSLLLRKKDSSRAVLSRAASPGKVLVPDGESDDLASPAQPEELQIPEDIEEQTAEVNMTGGTAEKLQSSEPTQGIVETITDGVTKGVKELVVGEKPRVVPKPGDGQKIYEIDPTLKDFRSHLDYRYSEYKRIRAAIDQHEGGLEAFSRGYEKLGFTRSAEGITYREWAPGAHSAALVGDFNNWNPNADTMTRDDYGVWEIFLPNNADGSSAIPHGSRVKIRMDTPSGVKDSISAWIKFSVQAPGEIPFNGIYYDPPEEEKYVFQHPQRKRPESLRIYESHIGMSSPEPKINSYANFRDEVLPRIKRLGYNAVQIMAIQEHSYYASFGYHVTNFFAPSSRFGTPEDLKSLIDRAHELGLLVLMDIVHSHSSNNTLDGLNGFDGTDTHYFHGGPRGHHWMWDSRLFNYGSWEVLRFLLSNARWWLEEYKFDGFRFDGVTSMMYTHHGLQMTFTGNYGEYFGFATDVDAVVYLMLVNDLIHGLYPDAVSIGEDVSGMPTFCIPVPDGGVGFDYRLHMAVADKWIELLKQSDESWKMGDIVHTLTNRRWLEKCVTYAESHDQALVGDKTIAFWLMDKDMYDFMALDRPSTLRIDRGIALHKMIRLVTMGLGGEGYLNFMGNEFGHPEWIDFPRGPQTLPTGKVLPGNNNSYDKCRRRFDLGDADFLRYRGMQEFDQAMQHLEEKYGFMTSEHQYVSRKHEEDKVIILKRGDLVFVFNFHWSNSFFDYRVGCSKPGKYKVALDSDDALFGGFSRLDHDVDYFTTEHPHDNRPRSFSVYTPSRTAVVYALTE

SEQ ID NO: 7 - DNA, 4431 bp, Triticum aestivum
atggcgtcgccggcattcgcagtttccgcggcgggcctcgcccggccgtcggctcctcgatccggcgggccagagcggagggggcgcggggtggagctgcagtcgccatcgctgctcttcggccgcaacaagggcacccgttcaccccgtaattattggcgctaccttcctcactcccattctcgtttattcgtagcgggctgcggttcagcgaccttacgttccctcctggtgtggtgatgtctgtaggtgccgtcggcgtcggaggttctggatggcgcgtggtcatgcgcgcgggtgggccgtccggggaggtgatgatccctgacggcggtagtggcggaacaccgccttccatcgacggtcccgttcagttcgactctgatgatctgaaggtagtttttatttctttccttgctagtaccttcctgcatgacaattgaaatctaagacaaaaacaccatatgcgaagcctacacggtaggttggtttacaactatgtgtgccacagttcgtctgaactttttgtccttcacatcgtgttaggttccattcatcgatgatgaaacaagcctacaggatggaggtgaagatactatttggtcttcagagacaaatcaggttactgaagaaattgatgctgaaggcacgagcagaatggacaaagaatcatctacgggagagaaattacgcattctgccaccaccgggaaatggacagcaaatatacgagattgacccaacgctccgagactttaagtaccatcttgagtatcggtatgcttcgcttctattgtgtgcactttaaactttaaatacaatttacagtctttgataagatgtgaatggctgcttgctgtgacacaaaactcttgaagttcgtagtcactcttgtgtgttcatggctctgaggtgacatggtaaccgaacaaaaataggaaagtggcaagaactgcaatgtgagctaccgataagcacccattgtaattgggtacactgattaatatatgtcttgatgggttctatgttttttcagtatctatgccaattgaacaacaatgccacttcatttcccctgtgttgcttttgtaaggatgaaacccatatgtccagatcaaactgtactagcagtctcactgtgccttaatggatcaaaaacagatacagcctatataggagaatacgttcagacattgatgaacacaaaggaggcatggatgtattttcccgcggttacgagaagtttggatttgtgcgcaggtgaaatttcttgactagataagtatgtatctaccttttttctgtatcgtatctacattcctcttcccatgcagcgctgaaggtatcacttaccgagaatgggctcctggagcagatgtatgttcttctgactgtctgatcgtttacctaagtatactagttctatctttcaactgcttgtgaataattagtgctcatctgctatcctaaggttggggattttgcacttcccagatgaacagcatattaagttgcacaactagctttatttagaactaactcttgcttccaattgcagtctgcagcattagttggcgacttcaacaattgggatccaaatgcagaccatatgagcaaagtatgcatgtagtttcacaaatatataattttttctttgtaaatttgtttcttaagatctgcttactatttaaatgtggttgaatatacaccttatatgtattccggagttgagctgtgaatatagttggaagtgtttaggagtattaaagtcactagactctattctttcacttgcctgttgcacgagcccattaattactagatatcaatgttgatgatgcttttgttgtataacgtcaaattgacaacatgcatgttacccttttatataagtaatgctgcacaaatatttttgatgatttagacatgatttaatgattttggttattgcaagacactgagcggttttacatagtaatggtattggagtaggctgactggataacccgtgaactgtagctccatgtggttgatatggatttacaaatgctcatattcaatttaattgttttcagaatgacttgggtatttgggagatttttctgccaaacaatgcagacggttcgccaccaattcctcacggctcacgggtgaaggttgttttcttctcctcgccaactgtgttaggctcaggaacatgttctgtattactcacaagctcttttgaacatctaggtgcgaatgggtactccatctgggacaaaggattcaattcctgcttggatcaagtactccgtgcagactccaggagatataccatacaatggaatatattatgatcctcccgaagaggtattttacttcgtcttctgtgcttttagatttcagatatttttaattggaaagaaaattatgatttgtttttctcacgaagcttcccaagtgttatttcaagttgttctacttcttatttgttgttggcatcttagttttctattcactaaccagttatgaaattcttacatgcatgtgcaggagaagtatgtattcaagcatcctcaacctaaacgaccaaaatcattgcggatatatgaaacacatgttggcatgagtagcccggtatttcatctttaccctgtattccataaatgaagttagctatatgcaattcaagttaatttacaatttgttacaatggtatttttgtgttgttggccttctttcgttttataagtaaaaagcttatcataaatttatgtgttatgccacttggttaatacaatctgaaaaatgtaactgtggacaatctagaactagataatacaaatctgaaaaaacatgctggaatagtgtcatttcagtcaaataggatgttttgaatgctcgagagaagtactagattgtgtagcatcaaaagctggtgtccatttgttcgaacgttttacttgatgtaactgtgaatgttacatcttttgctactaaagttcattttttcactatattacatgtttcatcaacaacttaattaacctcattccttacaaacatttgtatttacatttgttcctacataaatggttattttatatatcaacttatgaatcctgaacgttataattaagaccgatggtatatcaacgattgagataatttggcatatgcggatgaattttgtggcttgttatgctcttgttttaataatataataaatagattatgcttgttggtagcctttttacattaacacatgggcaattacttgtttctttgtgcaaccaggaaccaaagatcaacacatatgcaaactttcgggatgaggtgcttccaagaattaaaagacttgggtacaatgcagtgcaaataatggcaatccaagagcactcatactatggaagctttgggtagttctctgggtcgatttctgattcttttagttattttttgtccatggaacatatttcaactttagcaactatactattatattaacttttcagctattctcttccttttcttactagtaaagtatgtgtgtgcaatgcacgtattaggtaggatattagtggcacgttatattaggtaaaatatatttatggcacattgatatttgctaagatattaattgctttcttcgcgggaatggtaaaatattaattacatgacagatttcatgggatagcgttgagtctaaacatgtttataaccaatgatagtgatgggtaattagagcgttaaacatgtttggtgctcaacattggagcgatttgaactgctagattacatgatttgacggttgagatggtttggatctgcccctttgggtctttttgtattggtatagatgtgagagactgctgcttcttgctacttcctgtgttctcattctgagtagatatcttatgagtggacaactctatgtcgacattctggaagtatcactggttgatttggtctaaaataacatactgcacagatagccacataacagtgcgattacacacataatgaccatgtttgcatagagtggcggtagtatgttcctcaccatactagcataatgatttgttatataggagtatatcatattaacttcttttccaatgacatggaagctgtaacaactttcaaatcatatttgtcttttaagtgctgcttttttcctgtttgacaattaatacaataccacttttatgtgtttttacttctattgcaggtaccatgttaccaatttctttgcaccaagtagccgttttgggtccccagaagatttaaaatctttgattgatagagctcacgagcttggcttggttgtcctcatggatgttgttcacaggtacttaatgtaatttgccgttggcgtgttaggttcacattaatcttaattctttatttcaattcctatggcctctctcctagatggaacagtaaaagc

SEQ ID NO: 8 - protein, 416 aa, Triticum aestivum
MASPAFAVSAAGLARPSAPRSGGPERRGRGVELQSPSLLFGRNKGTRSPRAVGVGGSGWRVVMRAGGPSGEVMIPDGGSGGTPPSIDGPVQFDSDDLKVPFIDDETSLQDGGEDTIWSSETNQVTEEIDAEGTSRMDKESSTGEKLRILPPPGNGQQIYEIDPTLRDFKYHLEYRYSLYRRIRSDIDEHKGGMDVFSRGYEKFGFVRSAEGITYREWAPGADSAALVGDFNNWDPNADHMSKNDLGIWEIFLPNNADGSPPIPHGSRVKVRMGTPSGTKDSIPAWIKYSVQTPGDIPYNGIYYDPPEEEKYVFKHPQPKRPKSLRIYETHVGMSSPEPKINTYANFRDEVLPRIKRLGYNAVQIMAIQEHSYYGSFGYHVTNFFAPSSRFGSPEDLKSLIDRAHELGLVVLMDVVH

SEQ ID NO: 9 - DNA, 4727 bp, Triticum aestivum
gcctcctcatttcgctcgcgtgggtttaagcaggagacgaggcggggtcagttgggcagttaggttggatccgatccggctgcggcggcagcgacgagatggcgtcgccggcattcgcagtttccgcggcggggctcgcccggccgtcgactcctcgatccggcggggcagagcggagggggcgcggggtggagctgcagtcgccatcgctgctcttcggccgcaacaagggcacccgttcaccccgtaatttttggcgccaccttcctcactcccattctcgtttattcgcagcgggctgcggttcagcgatcttacgttccctactggtgtggtgatgtctgtaggtgccgtcagcgtcggaggttctggatggcgcgtggtcatgcgcgcgggtgggccgtccggggaggtgatgatccctgacggcggtagtggcggaacaccgccttccatcgacggtcccgttcagttcgactctgatgatctgaaggtagtttttcttttcctttttttgcatcgatctgaaggtagttgacatatattaccctgactaaactattactgccaccgtatttttatggttcgcttgaaatacctgtttacttgctacggtttgcactttcattgagacgtcagaagaaattcactgaattcctataatttggtagacaccgaaatatgtaccttttaggtcaaaatattccggcagttaagtttcagttgtatacaagaattcaaatatatatattttctcaaaatttacaactaattggtttagtttcaagtgaacgttttggtcctttggtcgagaagtaaaccgaaatcactgaaattcactgaatttcagtagtggccgaaacttttatagaactgaaattcaaaatctgctattcggcgaaattatatactaaagatttgcttatttcacacgtaggttgcggaatatcctctttctaatttgttggggaatggttcttattatcttgtcagtacctgcctgcatgacaattgaaatccaagacaaaacaccatatgcgaggcctacacgctaggttggttttacaactatgtgtgccacagttcttctgaactttttgtcttgcacattgtgttaggttgcattcatcgatgatgaaccaagcctacaggatgaaggtgaagatagtatttggtcttcagagacaaatcaggttactgaagaaattgatgttgaaggcacgaacataatggacaaagaatcatctacgggggagaaattacgcattgtgccaccaccaggaaatggacagcaaatatacgagattgacccaacgctccgagacttcaagtaccatcttgagtatcggtatgattcgcttctattgtgtgcactttaaaagaatttacagtcttcgctaagatgtgaatggctgcttgatgtatcacgaaattcttgaagttcatagtcactcttgtgtgttcatggttctgaggtaacttggtaaccgaacaaaataaggaaagtgcaagcactgcaatgtgagctactgataaccacccattgtaattgggtagactgattaatatatatgtcttcatgggctctatgtttcttttcaatatctatgccaattgaacaacaatgctttgtggacgggtgttcttttaccctctccttctatcaatagatgatacgcatactcatgcgtattctacaaaaaattgaacaacgatgccacttcatttcccccgtgttgcttttgtaaggatgaaacacatatgtccagatcaaactgtactagcagtctcactgtgccttaatggatcaaaaacagatacagcctatataggagaatacgttcagacattgatgaacacgaaggaggcatggatgtattttcccgcggttacgagaagtttggatttatgcgcaggtgaaatttcttgactaaataactatgtatctaccttttctttgtattgtatcaacattcctcttctcatgcagcgctgaaggtatcacttaccgagaatgggctcctggagcagatgtatgttcttctaaccatctgatcgtttacctaactatactagttctatctttcaactacttgtgaataattactgctcatcagctatcctaaggttggggattttgcacctcccagatgaacagcatattaagtcgcacaactagcattattaagaactaactcctgcttccaattgcagtctgcagcattagttggcgacttcaacaattgggatccaaatgcagaccatatgagcaaagtatgcatgtagtttcacaaataatattttctttgtagattagtttttttttagattggcctatctatttaaatgtggttgaatatacaccttatatgtattccagagttgagctgtaaatatagttggttggaagtgtttaggagtttaaattcactggactctattctttcacttgcctgttgcgcgagcccattactagatatcaatgttgatgatgcttttgttgtatgaggtcgaagtgaaacatgcatgttacccttttatataagtaaggttgcacatgtattttttatgatctaaacatcatttactgattttgttcttgcaagacattcagcagttttacataataatggtattggagtaggccgactgcatacctgaactgtagctccatgtggttgatatagatttacaaatgctcatattcaatgtaactgttttcagaatgacctcggtgtttgggagatttttctgccaaacaatgcagatggttcgccaccaattcctcacggctcacgggtgaaggttgtttttttctccttgccaaccgtgttaggctcaggaacatgtcttgcattactcagaagctcttttgaaaatctaggtgagaatggatactccatctgggataaaggattcaattcctgcttggatcaagtactccgtgcagactccaggagatataccatacaatggaatatattatgatcctcccgaagaggtattttacttcattttctgtgcttttagatttcagatatttttaattggaaagaaaattatgattttttttctcacgaagcttcccaattgctatttcaagctgtcctacttctatttgctgttggcatcttatttttctattcactaaccagttatgaaattccttacatgcatatgcaggagaagtatgtattcaagcatcctcaacctaagcgaccaaaatcattgcggatatatgaaacacatgttggcatgagtagcccggtatttcatctttaccctgtattccataaatgaaagttagctatatgcagtttaagttaatttacaggttgttacaatggtatttttgtgttgttgcccttctttcgttttataagtaaaaaacttatcataaatttatttgttatgccacttggttaatacaatctgaaaaatgtaactgtggacaatctagaactagataatacaaatctgaaaaaacaagctggaatagtgtcatttcagtcaaataggatgttttgaatgctcgagagaagtactagattgtgtagcatcaaaagctggtgtccatttggtcaaatgtttaacttgatgtaactgtgaatgttacatcttttgctactataagttcatatttttttcactatattacatgtttcatcaacaatttagttaacctaattccttacaaacatttgtatttaaatttgttcctacatgtatatttattttatatatcaacttataaatcctgaccgttataattaagaccaatggtatatcaatgattgagataatttggcatatgtggatgaattttgtggcttgttatgctcttgttttaataatataataaatagattatgcttgttggtagcctttttacattaacacatgggcaattacttgtttctttgtgcaaccaggaaccaaagatcaacacatatgcaaacttcagggatgaggtgcttccaagaattaaaagacttggatataatgcagtgcaaataatggcaatccaagagcactcatactatggaagctttgggtagttctctgggtcgatttctggttcttttagttattttttgtccatagaacatatttcaactttagcaactatactagtatattaacttttcagctattgtcttcctttttcttatgtgagagactgctgcttcttgctactttctgtgttctcattcagagtagacatcttatgagtggacaactctatgttgacattctggaagtatcactggttggtttggtctaaaataacatactgctcagatagccacataacagtatgattacacacacaatgaccatgtttgcatagagtggcggtagtatgttcctcaccatactagcataatgatttgttatataagagtatatcatattaacttcttttccaataacatggaagccttaacaactttcaaatcgtttttgtcttttaagtgctgcttttttcctgtttgacaattaatacaataccacttttatgtgtttctacttctattgcaggtaccatgttaccaatttctttgcaccaagtagccgttttgggtccccagaagatttaaaatcattgattgatagagctcacgagcttggcttggttgtcctcatggatgttgttcacaggtacttaatgtaatttgcggttggcgtgttaggttcacattaatcttaattctttatttcaattc

SEQ ID NO: 10 - protein, 415 aa, Triticum aestivum
MASPAFAVSAAGLARPSTPRSGGAERRGRGVELQSPSLLFGRNKGTRSPRAVSVGGSGWRVVMRAGGPSGEVMIPDGGSGGTPPSIDGPVQFDSDDLKVAFIDDEPSLQDEGEDSIWSSETNQVTEEIDVEGTNIMDKESSTGEKLRIVPPPGNGQQIYEIDPTLRDFKYHLEYRYSLYRRIRSDIDEHEGGMDVFSRGYEKFGFMRSAEGITYREWAPGADSAALVGDFNNWDPNADHMSKNDLGVWEIFLPNNADGSPPIPHGSRVKVRMDTPSGIKDSIPAWIKYSVQTPGDIPYNGIYYDPPEEEKYVFKHPQPKRPKSLRIYETHVGMSSPEPKINTANFRDEVLPRIKRLGYNAVQIMAIQEHSYYGSFGYHVTNFFAPSSRFGSPEDLKSLIDRAHELGLVVLMDVVH

SEQ ID NO: 11 - DNA, 14896 bp, Aegilops tauschii
  misc_feature (5)..(5): n is a, c, g, or t
  misc_feature (35)..(35): n is a, c, g, or t
  misc_feature (45)..(45): n is a, c, g, or t
  misc_feature (66)..(66): n is a, c, g, or t
  misc_feature (88)..(88): n is a, c, g, or t
  misc_feature (103)..(103): n is a, c, g, or t
  misc_feature (107)..(107): n is a, c, g, or t
  misc_feature (137)..(137): n is a, c, g, or t
  misc_feature (146)..(146): n is a, c, g, or t
  misc_feature (154)..(154): n is a, c, g, or t
  misc_feature (156)..(156): n is a, c, g, or t
  misc_feature (168)..(168): n is a, c, g, or t
  misc_feature (172)..(172): n is a, c, g, or t
  misc_feature (206)..(206): n is a, c, g, or t
  misc_feature (210)..(210): n is a, c, g, or t
  misc_feature (230)..(230): n is a, c, g, or t
  misc_feature (272)..(272): n is a, c, g, or t
  misc_feature (274)..(274): n is a, c, g, or t
  misc_feature (313)..(313): n is a, c, g, or t
  misc_feature (374)..(374): n is a, c, g, or t
  misc_feature (5514)..(5514): n is a, c, g, or t
  misc_feature (5541)..(5541): n is a, c, g, or t
  misc_feature (5574)..(5574): n is a, c, g, or t
  misc_feature (5586)..(5586): n is a, c, g, or t
  misc_feature (5602)..(5602): n is a, c, g, or t
  misc_feature (5619)..(5619): n is a, c, g, or t
  misc_feature (6366)..(6366): n is a, c, g, or t
  misc_feature (6596)..(6596): n is a, c, g, or t
  misc_feature (6604)..(6604): n is a, c, g, or t
  misc_feature (6623)..(6623): n is a, c, g, or t
  misc_feature (6676)..(6676): n is a, c, g, or t
  misc_feature (6746)..(6746): n is a, c, g, or t
  misc_feature (6787)..(6787): n is a, c, g, or t
  misc_feature (6803)..(6803): n is a, c, g, or t
  misc_feature (6845)..(6845): n is a, c, g, or t
  misc_feature (6864)..(6864): n is a, c, g, or t
  misc_feature (6877)..(6877): n is a, c, g, or t
  misc_feature (6963)..(6963): n is a, c, g, or t
  misc_feature (7055)..(7055): n is a, c, g, or t
  misc_feature (7123)..(7123): n is a, c, g, or t
  misc_feature (9161)..(9161): n is a, c, g, or t
  misc_feature (9206)..(9206): n is a, c, g, or t
  misc_feature (9284)..(9284): n is a, c, g, or t
  misc_feature (10857)..(10857): n is a, c, g, or t
  misc_feature (10861)..(10861): n is a, c, g, or t
  misc_feature (10926)..(10926): n is a, c, g, or t
  misc_feature (11177)..(11177): n is a, c, g, or t
  misc_feature (11224)..(11224): n is a, c, g, or t
  misc_feature (11336)..(11336): n is a, c, g, or t
  misc_feature (12749)..(12749): n is a, c, g, or t
  misc_feature (12771)..(12771): n is a, c, g, or t
  misc_feature (12964)..(12964): n is a, c, g, or t
  misc_feature (12984)..(12984): n is a, c, g, or t
  misc_feature (12986)..(12986): n is a, c, g, or t
  misc_feature (13126)..(13126): n is a, c, g, or t
  misc_feature (13893)..(13893): n is a, c, g, or t
  misc_feature (14086)..(14086): n is a, c, g, or t
  misc_feature (14109)..(14109): n is a, c, g, or t
  misc_feature (14156)..(14156): n is a, c, g, or t
  misc_feature (14173)..(14173): n is a, c, g, or t
  misc_feature (14517)..(14517): n is a, c, g, or t
  misc_feature (14591)..(14591): n is a, c, g, or t
ttttncggggttgcttcttccagattcatattcgnaaaatttcanatggagcttaaaaataatgtngttgagcttttttgagggtttncaaatggccaattanaacnttgggttttgaattaattgaatccaatttngaccaattnatttaagnanttttaaattggnatgnaaaacttttatttgaactattgtcgccttggaantttnattttttgagtttaaaaggncttgcgatatttttcttttgattgttttccaacccatgtaananagtgcgttaaaagagcaaaggtatacgccaaagaaggcncacccattacaaagccacataggcatgacccaactaaagaacccaaaccattgatgattcncaattaataaacccaccaaaatcagcttaaattagagcaagggcattacacatgcaacaaagtaggcaacattttcagtgcataagactacaatagacaacaacactatctcaacacgaccacgacaacggacaacatcgaataaaacccaaagaacacatgaagaaggcatgacgtcactgagcaaggaggctacaaatccaccaccgccgggccgacttgccaccaaggccatagaaggaccgtggggtgcataggcataaaccagagcaggaggcacatgaccaacaaagacaacatcaaccacgatcaagtaccacaacaggggaggagtgagggaaaatgccatcggagactcgaagtggacgttggagtatttttctttgattattttcaatattcaaactacacaagatcaacaacagatgagagaccaaaacatttgataactacagttggataatattggccatgatgtctgtttgatgatccgcccgagatgccaagctttgtagccttgcacgggctccccaacaaactgcctcactcgattgtcaaaaaagtaaaaatgattgtagaaaaaaaaactgactcactcgtcactaccctaccgtcctacatgacacctggccgcaagacgacgccgtcctcctgccgcgcgcgtccgcgatcacaccaccgcaaaaaccaaaacctcttcgccggtgcgtcccacgctaccatccatgcagccgtccgcccgcgcgcgcgttgcccgcaccacccgctggcggccaccacgccgccactctcgcgtgaaggctccgtccgcttcctcctagttccactctctctccgtgctagcagtatatagcatccgccctccgccccctcccaatcttagaacacccctccctttgcctcctcatttcgctcgcgtgggtttaagcaggagacgaggcggggtcagttgggcagttaggttggatccgatccggctgcggcggcggcgacgggatggctgcgccggcattcgcagtttccgcggcggggctggcccggccgtcggctcctcgatccggcggggcagagcggagggggcgcggggtggagctgcagtcgccatcgctgctcttcggccgcaacaagggcacccgttcaccccgtaattatttgcgccacctttctcactcacattctctcgtgtattctgtcgtgctcgcccttcgccgacgacgcgtgccgattccgtatcgggctgcggtgttcagcgatcttacgtcggttccctcctggtgtggtgatgtctgtaggtgccgtcggcgtcggaggttctggatggcgcgtggtcatgcgcgcgggggggccgtccggggaggtgatgatccctgacggcggtagtggcggaacaccgccttccatcgacggtcccgttcagttcgattctgatgatctgaaggtagttttttttttgcatcgatctgaaggtacttgacatatactactgtattaccctgagtaaatactgccaccatatttttatggttcgcttgaaatacctgtttacttgctacggttttcactttcattgagacgtcggacgaaattcactgaattcctataatttggtagacaccgaaatatatactactccttccgtcccataatataagagcgtttttggcaccttatattatagggcggagggagtaccttttaggtcaaaatattgtggtagtttcaattgtatacaagaattcaaatattttttttaaaaaaaaatcaactaattggttgagtttcaagtgaagcgttttggtcctttggctgagatgtaaaccgaaatcactgaaattcatagtagccgaaactttaatagaactgaaactcaaaatctgctatccggcgaaattctaaagatttgcttatttcacacgtaggttgcagtacaccctctttctaatttattggggaaggggtattattatcttgttagtacctgcctgcatgacaattgaaatctaagacaaaacaccatatgcgaggcctacacacggtaggttggtttacaactatgtgtgccacagttcgtctgaactttttgtccttcacatcgtgttaggttccattcattgatgatgaaacaagcctacaggatggaggtgaagatagtatttggtcttcagagacaaatcaggttagtgaagaaattgatgctgaagacacgagcagaatggacaaagaatcatctacgagggagaaattacgcattctgccaccaccgggaaatggacagcaaatatacgagattgacccaacgctccgagactttaagtaccatcttgagtatcggtatgcttcgcttctattgtgtgcactttaaaaacaatttacagtctttgataagatgtgaatggctgcttgctgtgacacgaaactcttgaagttcgtagtcactcttgtgtgttcatggttctgaggtaacatggtaaccgaacaaaaataggaaagtggcaagcactgcaatgtgagctactgataaccacccattgtaattgggtacactgattaatatatatgtcttcatgggctctattttttttcaatatctatgccaattgaacaacaatgctttgtggacgggtgttcttttaccctcttcttctatcaatagatgatatgcatactcatgcgtatcctacaaaaaattgaacaacaatgccactttcccccgtgttgcttttgtaaggatgaaacacatatgtccagatcaaactatactagcagtctaactgtgccttaatggatcaaaaacagatatagcctatacaggagaatacgttcagacattgatgaacacgaaggaggcatggatgtattttcccgcggttacgagaagtttggatttatgcgcaggtgaaatttcttgactaaataactatgtatctaccttttctttgtactctatcaacattcctcttcccatgcagcgctgaaggtatcacttaccgagaatgggctcctggagcagatgtacgttcttctaaccatctgatcgtttacctgactatactaattctatctttcaactaattgtgaataattactgctcatcagctatcctaaggttggggattttgcacctcccagatgaacagcatattaagtcgcacaactagcattattaagaactaactcctgcttccaattgcagtctgcagcattagttggcgacttcaacaattgggatccaaatgcagaccatatgagcaaagtatgcatgtagtttcacaaatatatcatattttctttgtagatttttttttttagatcggcttatctatttaaatgtggttgaatatacaccttatatgtacgttgagctgtaaatatagttggaagtgtttaggagtattaaattcactggactctattctttcacttgcctgttgcacgagcccattactagatatcaatgttgatgatgcttttgttgtatgaggtcgaagtgaaacatgcatgttacccttttatataagtaaggttgcacatgtattttttatgatctaaacattatttactgattttgttcttgcaagacactaagcagttttacataataatggcgttggagcaggccgactgcacatctgaactgtagctccatgtggttgatatagattacaaatgctcatattcaatgtaactgttttcagaatgaccttggtgtttgggagatttttctgccaaacaatgcagatggttcgccaccaattcctcacggctcacgggtgaaggttgttttcttctccttgccaacggtgttaggctcaggaacatgtcctgtattactcagaagctcttttgaacatctaggtgagaatggatactccatctgggataaaggattcaattcctgcttggatcaagtactccgtgcagactccaggagatataccatacaatggaatatattatgatcctcccgaagaggtattttacttcatcttctgtgcttttagatttcagatatttttattagaagaaaattatgattttttccctcacgaaccttcccaattgctatttcaagctgtcctacttatttgctgctggcatcttatttttctattctctaaccagttatgaaattccttacatgcatatgcaggagaagtatgtattcaagcatcctcaacctaaacgaccaaaatcattgcggatatatgaaacacatgttggcatgagtagcccggtatttcatctttaccatgtattccataaatgaagttagctatatgcagttcaaatttatttacaggttgttacaatggtatttttgtgttggtgcccttctttcgttttataagtaaaaaacttatcataaatttatttgttatgccgcttggttaatacaatctgaaaaatgtaactgtggacaatctagaactagataatacaaatctgaaaaaacatgctggaatagtgtcatttcagtcaactaggatgttttgaatgctcaagagaagtactagtgtgtagcatcaaaagctggtgtccatttgttcaaatgtttaattaacactatagtgaaaacaagtaattgcacaaagaaacaagtaattgcccaagttcatatgttttttcactatattacatgtttcatcaacaatttaattaacctcattccttacaaacatttgtatttacatttgttcctacatatatagttattttatatatcaactttataaatcatgactgttataattaaaaccgatggtatatcaacgattgagataatttggcatatgtggatgaattttgtggcttgttatgctcttgttttaataacataataaatagattatgcttgttggtagcctttttacattaacacatgggcaattacttgtttctttgtgcaaccaggaaccaaagatcgacacatatgcaaacttcagggatgaggtgcttccaagaattaaaagacttggatacaatgcagtgcaaataatggcaatccaagagcactcatactatggaagctttgggtagttctctgggtcgatttctggttcttttagttatcttttgtccatagaacatatttcaactttagcaactatactattatattaacttttcagctattgtcttnctttttcttatgtgagagactgctgcntcttgctacttcctgtgttctcattcagagtanacatcttatgantagacaactctatgtngacattccggaagtatncactggctgattcggtctaaaataacatactgctcagatagccacataacagtacgattacacacataatgaccatgtttgcatagagtggcggtagtatgttcctcaccatactagcataatgacttgttatataagagtatatcatattaacttcttttccaatgacatggaagctgtaacaactttcaaatcatttttgtcttttaagtgctgcttttttcctgtttgacaattaatacaataccacttttatgtgtttttacttctattgcaggtaccatgttaccaatttctttgcaccaagtagccgttttgggtccccagaagatttaaaatctttgattgatagagctcacgagcttggcttggttgtcctcatggatgttgttcacaggtacttaatgtaatttgaggttggcgtgttaagttcacattaatcttaattctttatttcaattcctatggcctctctcctagattggaacagtaaaagcatcatccagtttgtataaattgctaaaagaacattttacatgttaagtattttcaattactatgaaacatataaatttacatacttattgattttacgacagaagtaccgatctcacaagatgaacaattggttgatcacatatcatttcatactacaatacaagaaaatgaatagagaacgagttaatattagccttggtaaaatcagcaacttgtttggaaataaagtatagtgatgccagtgcaaanaacaaggcatcaagttggtttcagctcccacggtcggtgctagctgtcaagggtaatttgcacgtagtcgcacatagatttgtgtgggagtggaaagtaaccacagattgtccgaggaacacgggacacacgtcttagccacaggtttgggctccccttgatgcgggtagtagctttactccttatatgaaattatctcaagatagatttcaatttggggttacacttangaactcancaagttaaggatcaactcnctgagttctatacgactgatctttgaccgagatatcttgatcaggctaagtancaaaatccaggccttgagatgttgaacatgtccttcattttgggctgggtgcccttgggcataaggtgtngtccttccttcatgtgcttcttgcagcgtatgacataaacntcctctgagttggtanatgcacggttccctttgaggaaatcaggggtagtcgcatctngggaaagttggtcacccangcatggatcctcngcgcacaccgggcaaacacggtgaaaccacttctcctcgacactagctaacttgacattcaagcaaactaagaatataactttatntctaaatgaaccggacaccctccttgtgcctgcacctacagagtacaatgccagttttggactgaactcttgtgttcatgtatgtgctaatnacataggttctaaccatgattctaaatagcgcgttataactccactatagtaatgctatagcgtttanaagatcccgcactaagggaccttagtccaaatacatgatcaaacattttacatagcgcgctatagctatttaaaactatggtcacccgctaagaggcataactcgctatttaaaactatggttctaacttttaatctattttatgtcttggtccaaagcccctttttgttctatagctttacctttgggttgagatcacccttaacccattggtaatcctggttgatttactccatcctttcttgcgtagctttacttttggttttttgtttctcacagtcacgcgtcaaataataccttggacgggttgaatggttttgatggcacggatacacattacttccatggcggttcacggggccatcactggatgtgggattcccgtgtgtttaactatgggaataaggaagtatgggactatagaatttctattgccatttgttatgtatttatccattaattaatcctccaaccgatattccaacattgttatctttatacaggttataaggtttctactttccaatgcaagatggtggctagaggagtataagtttgatggtttccgattcgatggcgcgacctccatgatgtatacccatcatggattacaagtaattcattgcttgattgtctttgttctatcttgactacctgtgcaactttaataagattacgcctagctaatattttcttttatgttatagtatcaatttttatttgagcttgaaacctaaattactttttttttgaattgctgcgctctattttaggtaacctttacaggaagctaccatgaatattttggctttgccactgatgtagatgcggtcgtttacttgatgctgatgaatgatctaattcatgggttttatcctgaagccgtaactatcggtgaagatgtaagtgtttctatagtcatctttcaatatgaatttgttagaactattggtacttatcttttttgtagtttaggctattctgttcattcttacaggaggtgcatacagaagttgctttagattttgaaacgcagtgcacattgtgccattactttgtagctatatcgagttgagacttgagagccatggtaatcaagttcctgacgtggcattgcattagatagttgcatgtctaagttcctgacgtggagatagaagaaagaacgcaccccccgcgtcgctcctctcagggcgacacgggcggagccctcacccccgccgccacagggagcatccacccttctcctctcccctcgccgccgccggagggcaaagaccgcgcggcgtcgcggcggtgggtgcggcctgggctggcatctggcagcggcgatttggcctcccctgcccagaactgtgctgccgcggtttgtggcagcttgggcatcggcagtggcccgagtctgcggtggcggcgtgtctggcgtccggaggtgcagcgattgtgcggttgtgtggctcaggctcggagggcgtgcgggctgccaggtccggccagatctggcctcgagtggcttcgtacggggcggtggctgttgcgggtccgtgggccgaggttcgggtgtggctgctgcttgcccggaccggtggtgcgtaacgatgccggagcagcgtcctcgggtcgttgaagtgggcgctcctccggcagcttcaggtggtgattcgtcgcagcgggtggtgcactgggggtctcggctgattgtggtgccatggtggtggtggttgttggcggtagcaaagtgcctggtgcacacggctagggttttggcggatggacagacttgatgcaatgccttagggcatagtgaatttcagctaagtacctagcaccgaccttggtcaatgccgccgccgctggtgtcttaggacgttgttgcccttgttggaggcgtgttgtggagccccttcacctccatgggcatttagatctcgagctctctgggtgaaaacgccggctttggctttggccggagtgggcggtggcggcgtaaccgtcgctccccccatgggggtgtagtcttggaggtctagacttctgntaagcgtcagtggttggtgtggtcctgaaggttcgtatcggctangcaggagcacggtctcagggccggtgtggaagccagagcagcagctccggagagcgcatttgtgttgcatggtgcccnagtctggtcgcttgggtggcttgaacccatccggttcagtgggtacacagccttggggctggtgtgtggagaacgcctttatgttatagggtatcaattttgttcacttgggttacggagtcgtcgactcgtctggtacacggcctcagggccgatatgtgtctctctgtgtgtgtctgtttgtgtgttgttgaggtttgtacgccagggcggcggctccaagtcgtgttgtatggtatcgactctggtcgttagagcgactgagtcgccggctcatttggggcgcagcctcggaactggtgtgtgtgtcacaggctcacaactgtattagttttgagctagttttccttgttaaccggtcaattaaaattcttctgtatgaaaaggcagagctactgtcagttactagggaaaaaatgtttctggcatggaaaactattttctatccatttcatgtagtgacaacttttctttttcttgagtgagactactaactttccatgaaagtcagatgaaaatcaacaacttctataaacaaacagaactttccagaaataaggaacaaattgttggatatatcagcaatttttcaatttatttatttaatacgaaagcatgatgatagtgctggcaagatttaatcctaattgtaatctaaacatgtgagtgcgtgcataaaacatgcatatctcttaacatagtgagtactggaaactcatgaaccaagcagaagtgggatgaatggatcataccctccagtagcaaaagtaaggggttagggccgtggcaacagcagcattggcattggtggccttcttcaaggaaccattgttcccacccatgggtttggttggggaagtcaagaaagtagtcgaagtcgtggatgcaaaaggacagaagggagccgtcagggtgacatgctccccaataaccttattgatctccacctggtgcatggttctgttgcgtgccgcagagaaggtgcgcacatgtacccactcctcttctcatgctcccaatgggtcatgaagagagttcttatatattggtccaaattctcctccactccttgggtcggactaaatttccaaccatttcatgaaaccactaatgggtctttgagattatgcaggaattattaattatataatatggcccaaggcccatctaactttcaacaataataacttaattgttcaactgaggtgttggtttttcatttgaattctcaggttagtggaatgcctacatttgcccttcctgttcaagttggtggggttggttttgactatcgcttacatatggctgttgccgacaaatggattgaacttctcaagtaagtgtttcaaaattggtatgcatatgttaatattttactggacagaagatttgattgtcagtgtatattaatgcaattaaaatgttcctttgcgtaacactattgcacatatggacttccacatgaatgtccaaaaacatgtatcgttattagtgtatttgatttggccacaatgtgattatagttgtgatttcgtagtttatacagtataacaacaaaagtaggatacatgtnccancttttgggaattcttataatgatattacacttttttaatcttgcatccctcatcatttctattgnctcagttgtttcaagtttctataaaagtttggtttcgtgttctggttattgatgtggagtatcttgtatctgaaacatgaattgcaactttttattctaaacagaggaaacgatgaagcttgggagatgggtaatattgtgcacacactaacaaacagaaggtggctggaaaagtgtgttacttatgctgaaagtcacgatcaagcacttgttggagacaagactattgcattctggttgatggacaaggnaacaacacattatttctccagactttaaatactaacatttattttgnttcgcaatttccttatatctatgatttttaattatacttatctctcttgattttcctccccacaaaaatgcaagctagaatttttttcctcatgaaagtatgcaaagcttgngcctatgcattgataaagtatttacaagcctaagaataggcgacaaccgaccactcaagcgaagtccacaatcaaatggttgtcagacacgttaccgaactacttttagcctaaatgacaaccacacaaacacactgggttgcccttgctttggataaatcgatggcccctagactgccggtcgcacctcggaactgccaaccgccatggccgcttgaatagtgaaccatcacacattgccatatcctctacatgttgaaacttagtacgcaaccgtagtcgatcgtgcccccaagatgccacatcacgggattggcacatggctgatgcaagtaggaaccactgaaaaagccaaggcttgtgttcataccaatcgaaggaaaaccttgaagaacaaagccattagaaaggtatcaacatcaactggctacctcgtctgatctaggtctgaatcgacaaacccgatttggcttttcactctaaggattagacaacaggggatggggtaaattggtattccttgacaatgcccccaaggtggaaacggtgttaggaaggcgtcactagtccttttatacagactgctaagtgcggagacgggaatcgaacccgtgacctcaaggttatgagcctcgtcggcattgacagtgggaatatcaagtgcccctaacacttaggtgttcccatgtctagaaaaatcaattttaaatgtttcaaaaaaaatctttttttgtgaatcttcataaaacatgtgtttgcaacccctaaaaagtacaaatccaaactcagaatacatataggacaacacaaaagacaaatctagatgtgaacattgccatttttgttttttgattctattcatgatgatttgtctttttcgttcctccaagtattttgattttaattttttagaggtcgtagacacatcctatgaactttcacaactctttttctagaatcgtttgaaacgtttaaaaatgaatctctagatatggggaatgacaacgcccaagtgttgggagcactatttttttttcccacacctacctggtggggatgggtttcgtttgaagccgcatgaccaccactcatgccatgggtgcagccccatgaaggctcctcaacaaaatgtatcaccacccgcaatcacactagctcgacagcctgattgccatgccatcccaccaacaaggactaccatgcattgcacatcaggaccaacatagactgactgcaaggagctggaacatggtttaggagcctatgtacttgaaacctatacctgcagtgagatgcccggacctacgacaacaccactagagcacacatcagcaaccctgggcaaagcatgacaaatgatgccaggtacatccatccgtagatgttgcaagatgacgccggacgggaactaanagcatcttcaataacttgtggnatgttagtttgttacaaaatatagtaatctcttcaccaataagccattctacaaatactccaatggagtgtatttagcttgtcgaataggaggtgagagaatatataggattgctcttaggtatcgctaagtgatgtaagcgcaagccctatggttgtcccaatcttcataatttgtaggtggcaaaggggancatcacaaagaacacatagncntaaagaggaaacacccaaacaatattctcatcacacatgtcctctttagtttaatgctttgctaaccctaatttgagtccatggtacagtttatacagcatagggacgaagctggtaggtaggagagggatacatggccncttgactcgatttccacgcaggcatgggacgggcagtccaggttgcaagcctgacagtctggtcgttgtagctcgtccggatcagggcttccccatgcgccgctcgaagggctcactccaggtgtcgatagtctaggctccaagttggacagccggcttcaccaatttagcttttgttgcctagcgtgtggtagccggactaaggaccagacggtgttctagagaaggtttttgtctggttgttggattccagtagcccatctccttcgtcgtgcacttcctccttcgcttccacgcttccttcgcagatggtgtaggcgtactcttgtgcttgccttggtaaattcgctctcatgttcaatatggacgaactcattgccacacgccgccatgtttgaagggtaagtcccatgctcaaccatctcatcaccgttgccaaggatgaaggccatatggtgtggctcatcatcatcatccgcctccatgactgaagggaatatcccatgctcaaccatctcacttgaggtgcctccgaagatggagcggtcacacttgcttgttgttggtgatcgacgtgatgtagtcgccggagcgtcagagcttgaaggagtatcacttatttgtaactcgaggaagagaaatgttgcttgatgtagcattgtgtccattgttggtgtagattcttcaaggaatgttttcttgtaggctttatgcatcgttttcttgatgtcgtggccattcctcttcatgatgcgtttggagtgtgnaagcgctcttcttgttgatgatgttcacggtcaagggtgtggccttggaatccatcgttgcgaagaaggttgtagcttgatgttgctcttgtactttgaggtgtcaatgccggtgtgatcctgaagacttgtggtggttgagcacgttttgaaagagttgtgcgtcaatcttggcgtcccaatggtccatctnggcgtcaaagtttttggtgtagncctagaccggaggtgatgtgccttctctattcatattgacactcgancaaagtgtgagtggacnaagggaaagaacaataccaaagttacctctttccgatgttggtgaaggatcaagcgatctcacactatggaatattaagagagaacaataccaaagttacctctttccgatacattcgtcaacacaatacctttgtcgaggttggaggcaaccggccttgatttcggttgtggtgtcaaaggatggagtggttgttgttgttacgagaaccaaagcggaagaacaaccacaaatcaaaaaaggggcgaaagatgacaaatttcagcagattcggaagaggtcggacagtcgagttggtggcccctttttcgactcgagcaaagtgtgagtggcaagggaaagancaataccaaagttacctctttccgatgttggtgaaggatcaagcgatctcacactatggaatattaagagagancaataccaaagttacctcttcccgatacattggtcaacacaatacctttgtcgaggtcagaggcaaccggccttgctttcggttgtggtgtcaaaggatggagtggttgttgttgttacgagaaccaaagcggaagaacaaccacaaatcgaaaaaggggcgaaagatgaacaaatttcagcagattcaagagaggtcggacagtccgagttggtggccggacgggggttggctggacagtccgggttggaagctgacagttcgggtaggtcaactcggctgttcttcaggggaaattggatcga

SEQ ID NO: 12 - protein, 623 aa, Aegilops tauschii
MAAPAFAVSAAGLARPSAPRSGGAERRGRGVELQSPSLLFGRNKGTRSPRAVGVGGSGWRVVMRAGGPSGEVMIPDGGSGGTPPSIDGPVQFDSDDLKVPFIDDETSLQDGGEDSIWSSETNQVSEEIDAEDTSRMDKESSTREKLRILPPPGNGQQIYEIDPTLRDFKYHLEYRYSLYRRIRSDIDEHEGGMDVFSRGYEKFGFMRSAEGITYREWAPGADSAALVGDFNNWDPNADHMSKNDLGVWEIFLPNNADGSPPIPHGSRVKVRMDTPSGIKDSIPAWIKYSVQTPGDIPYNGIYYDPPEEEKYVFKHPQPKRPKSLRIYETHVGMSSPEPKIDTYANFRDEVLPRIKRLGYNAVQIMAIQEHSYYGSFGYHVTNFFAPSSRFGSPEDLKSLIDRAHELGLVVLMDVVHSHASNNTLDGLNGFDGTDTHYFHGGSRGHHWMWDSRVFNYGNKEVIRFLLSNARWWLEEYKFDGFRFDGATSMMYTHHGLQVTFTGSYHEYFGFATDVDAVVYLMLMNDLIHGFYPEAVTIGEDVSGMPTFALPVQVGGVGFDYRLHMAVADKWIELLKGNDEAWEMGNIVHTLTNRRWLEKCVTYAESHDQALVGDKTIAFWLMDK

SEQ ID NO: 13 - DNA, 23 bp, Artificial Sequence
  Synthetic Construct
acggctttgatcatctcctccca

SEQ ID NO: 14 - DNA, 25 bp, Artificial Sequence
  Synthetic Construct
tttgtctctttgatgttccccaaat

SEQ ID NO: 15 - DNA, 31 bp, Artificial Sequence
  Synthetic Construct
tatgaccagagtatgtctacagcttggcaat

SEQ ID NO: 16 - DNA, 27 bp, Artificial Sequence
  Synthetic Construct
tgcatcctaagtgggaaaccctaacca

SEQ ID NO: 17 - DNA, 27 bp, Artificial Sequence
  Synthetic Construct
tcaatttggatcagaggggatagtcca

SEQ ID NO: 18 - DNA, 27 bp, Artificial Sequence
  Synthetic Construct
tgacaaggttgcccatttctaatgcaa

SEQ ID NO: 19 - DNA, 28 bp, Artificial Sequence
  Synthetic Construct
gatagctggattaggcgatcgcctcagg

SEQ ID NO: 20 - DNA, 30 bp, Artificial Sequence
  Synthetic Construct
ttggtagaggaattagcaaagtaaaatcca

SEQ ID NO: 21 - DNA, 32 bp, Artificial Sequence
  Synthetic Construct
ggtagaaccttttgcattatgtgtgcttttcc

SEQ ID NO: 22 - DNA, 33 bp, Artificial Sequence
  Synthetic Construct
gctacctcgaaatgcaatggaaatcttagagac

SEQ ID NO: 23 - DNA, 27 bp, Artificial Sequence
  Synthetic Construct
ccaaggagggagtgaggagcttgactt

SEQ ID NO: 24 - DNA, 27 bp, Artificial Sequence
  Synthetic Construct
tgtcagcttgaatgcccttgcacttct

SEQ ID NO: 25 - DNA, 23 bp, Artificial Sequence
  Synthetic Construct
gatcgcgcttcctgaacctgtat

SEQ ID NO: 26 - DNA, 25 bp, Artificial Sequence
  Synthetic Construct
ctcagaccacgaagggatctgtatg

SEQ ID NO: 27 - DNA, 27 bp, Artificial Sequence
  Synthetic Construct
atgaatacgtgcaacactcccatctgc

SEQ ID NO: 28 - DNA, 29 bp, Artificial Sequence
  Synthetic construct
ggaagcaaagttttgcacttgccaatatg

SEQ ID NO: 29 - DNA, 28 bp, Artificial Sequence
  Synthetic Construct
cgtctccagcaagccatttcctacctta

SEQ ID NO: 30 - DNA, 28 bp, Artificial Sequence
  Synthetic Construct
ttttgccactagtttttgccaattttcc

SEQ ID NO: 31 - DNA, 29 bp, Artificial Sequence
  Synthetic Construct
tcaatcaatttggatcagagggaacatca

SEQ ID NO: 32 - DNA, 36 bp, Artificial Sequence
  Synthetic Construct
tagcagtgcaggaatttaagttaaaccactattaca

SEQ ID NO: 33 - DNA, 24 bp, Artificial Sequence
  Synthetic Construct
ctcccattctcgtttattcgtagc

SEQ ID NO: 34 - DNA, 26 bp, Artificial Sequence
  Synthetic Construct
gttcggttaccatgtcacctcagagc

SEQ ID NO: 35 - DNA, 28 bp, Artificial Sequence
  Synthetic Construct
gccaattgaacaacaatgccacttcatt

SEQ ID NO: 36 - DNA, 24 bp, Artificial Sequence
  Synthetic Construct
gagtacccattcgcacctagatgt

SEQ ID NO: 37 - DNA, 27 bp, Artificial Sequence
  Synthetic Construct
gcctgttgcacgagcccattaattact

SEQ ID NO: 38 - DNA, 28 bp, Artificial Sequence
  Synthetic Construct
ttcgaacaaatggacaccagcttttgat

SEQ ID NO: 39 - DNA, 28 bp, Artificial Sequence
  Synthetic Construct
ttatatatcaacttatgaatcctgaacg

SEQ ID NO: 40 - DNA, 31 bp, Artificial Sequence
  Synthetic Construct
gtaaagtgttcttttagcaatttatacaaac

SEQ ID NO: 41 - DNA, 30 bp, Artificial Sequence
  Synthetic Construct
gcctcctcatttcgctcgcgtgggtttaag

SEQ ID NO: 42 - DNA, 36 bp, Artificial Sequence
  Synthetic Construct
agtgactatgaacttcaagaatttcgtgatacatca

SEQ ID NO: 43 - DNA, 32 bp, Artificial Sequence
  Synthetic Construct
ctacaaaaaattgaacaacgatgccacttcat

SEQ ID NO: 44 - DNA, 27 bp, Artificial Sequence
  Synthetic Construct
ccaactatatttacagctcaactctgg

SEQ ID NO: 45 - DNA, 27 bp, Artificial Sequence
  Synthetic Construct
actgattttgttcttgcaagacattca

SEQ ID NO: 46 - DNA, 24 bp, Artificial Sequence
  Synthetic Construct
caaatggacaccagcttttgatgc

SEQ ID NO: 47 - DNA, 37 bp, Artificial Sequence
  Synthetic Construct
aaagttagctatatgcagtttaagttaatttacaggt

SEQ ID NO: 48 - DNA, 30 bp, Artificial Sequence
  Synthetic Construct
tgtaagatgttctttcagcaatttatacta

SEQ ID NO: 49 - DNA, 22 bp, Artificial Sequence
  Synthetic Construct
acgacgcgtgccgattccgtat

SEQ ID NO: 50 - DNA, 35 bp, Artificial Sequence
  Synthetic Construct
gccattcacatcttatcaaagactgtaaattgttt

SEQ ID NO: 51 - DNA, 34 bp, Artificial Sequence
  Synthetic Construct
atcctacaaaaaattgaacaacaatgccactttc

SEQ ID NO: 52 - DNA, 25 bp, Artificial Sequence
  Synthetic Construct
acatggagctacagttcagatgtgc

SEQ ID NO: 53 - DNA, 27 bp, Artificial Sequence
  Synthetic Construct
gcctgttgcacgagcccattactagat

SEQ ID NO: 54 - DNA, 34 bp, Artificial Sequence
  Synthetic Construct
ggcaattacttgtttctttgtgcaattacttgtt

SEQ ID NO: 55 - DNA, 28 bp, Artificial Sequence
  Synthetic Construct
gttttgaatgctcaagagaagtactagt

SEQ ID NO: 56 - DNA, 30 bp, Artificial Sequence; identical to SEQ ID NO: 48
  Synthetic Construct

SEQ ID NO: 57 - DNA, 28 bp, Artificial Sequence
  Synthetic Construct
ttatgtcttggtccaaagcccctttttg

SEQ ID NO: 58 - DNA, 30 bp, Artificial Sequence
  Synthetic Construct
tccacgtcaggaacttagacatgcaactat